European Patent Specification EP 3 884 024 B1, published August 7, 2024. Title: Detergent Composition. Applicant: Unilever. The sequence listing filed with the application follows.

SEQUENCE LISTING (2 sequences)

SEQ ID NO: 1 - protein, 157 aa, Corynebacterium
MNLALSGTFFNVNIRHLEGDGFSLFVDSDKKGEEDVPTARLKMEHAVASDLCLYVTTDLPAVGESTLALKAKGDNSVEATGLLVGASNIEGSLVMQDANVGIDASQLSQSADPGTWGLYAKQVSLTADDVRATSLGAKTLSAKNVGVSVERGRGNVC

SEQ ID NO: 2 - protein, 190 aa, Corynebacterium
MGRINVPKAAVGLVAGFAAFGVAGVAVAQGGLTANLALSGTFFNVNIRHLEGDGFSLFVDSDKKGEEDVPTARLKMEHAVASDLCLYVTTDLPAVGESTLALKAKGDNSVEATGLLVGASNIEGSLVMQDANVGIDASQLSQSADPGTWGLYAKQVSLTADDVRATSLGAKTLSAKNVGVSVERGRGNVC